European Patent Application EP 4 194 568 A1, published June 14, 2023. Title: COVID-19-associated Venous Thromboembolism. Applicant: GENINCODE UK Limited. The sequence listing filed with the application follows.

SEQUENCE LISTING (25 sequences)

SEQ ID NO: 1 - DNA, 15 bp, Homo sapiens
  rs1801020 risk allele
ggacggatgccatga

SEQ ID NO: 2 - DNA, 15 bp, Homo sapiens
  rs1801020 non-risk allele
ggacggacgccatga

SEQ ID NO: 3 - DNA, 15 bp, Homo sapiens
  rs8176719 risk allele
ctcgtggtgacccct

SEQ ID NO: 4 - DNA, 15 bp, Homo sapiens
  rs8176719 non-risk allele
ctcgtggtacccctt

SEQ ID NO: 5 - DNA, 14 bp, Homo sapiens
  rs7853989 risk allele
ggaggtgcgcgcct

SEQ ID NO: 6 - DNA, 14 bp, Homo sapiens
  rs7853989 non-risk allele
ggaggtgggcgcct

SEQ ID NO: 7 - DNA, 17 bp, Homo sapiens
  rs8176743 risk allele
tgcaccccggcttctac

SEQ ID NO: 8 - DNA, 17 bp, Homo sapiens
  rs8176743 non-risk allele
tgcaccccagcttctac

SEQ ID NO: 9 - DNA, 16 bp, Homo sapiens
  rs8176750 risk allele
tccggaacccgtgagc

SEQ ID NO: 10 - DNA, 16 bp, Homo sapiens
  rs8176750 non-risk allele
tccggaaccgtgagcg

SEQ ID NO: 11 - DNA, 17 bp, Homo sapiens
  rs2232698 risk allele
cctgctgtgaaagatct

SEQ ID NO: 12 - DNA, 17 bp, Homo sapiens
  rs2232698 non-risk allele
cctgctgcgaaagatct

SEQ ID NO: 13 - DNA, 18 bp, Homo sapiens
  rs121909548 risk allele
cggtacttgaagctgctt

SEQ ID NO: 14 - DNA, 18 bp, Homo sapiens
  rs121909548 non-risk allele
cggtacttgcagctgctt

SEQ ID NO: 15 - DNA, 15 bp, Homo sapiens
  rs6025 risk allele
attccttgcctgtcc

SEQ ID NO: 16 - DNA, 15 bp, Homo sapiens
  rs6025 non-risk allele
attcctcgcctgtcc

SEQ ID NO: 17 - DNA, 19 bp, Homo sapiens
  rs118203906 risk allele
gaaaaccacgaatcttaag

SEQ ID NO: 18 - DNA, 19 bp, Homo sapiens
  rs118203906 non-risk allele
gaaaaccaggaatcttaag

SEQ ID NO: 19 - DNA, 19 bp, Homo sapiens
  rs118203905 risk allele
aagaaaaccgggaatctta

SEQ ID NO: 20 - DNA, 19 bp, Homo sapiens
  rs118203905 non-risk allele
aagaaaaccaggaatctta

SEQ ID NO: 21 - DNA, 16 bp, Homo sapiens
  rs5985 risk allele
gggcaccacgccctga

SEQ ID NO: 22 - DNA, 16 bp, Homo sapiens
  rs5985 non-risk allele
gggcaccaagccctga

SEQ ID NO: 23 - DNA, 17 bp, Homo sapiens
  rs1799963 risk allele
tctcagcaagcctcaat

SEQ ID NO: 24 - DNA, 17 bp, Homo sapiens
  rs1799963 non-risk allele
tctcagcgagcctcaat

SEQ ID NO: 25 - DNA, 53 bp, Homo sapiens
  rs8176749 risk allele
gagcaccttggtgggtttgtggcgcagcaggtacttgttcaggtggctctcgt